European Patent Application EP 4 491 632 A1, published January 15, 2025. Title: 一种靶向ROR1的结合分子及其应用. Applicant: SANYOU BIOPHARMACEUTICALS CO., LTD. The sequence listing filed with the application follows.

SEQUENCE LISTING (125 sequences)

SEQ ID NO: 1 - protein, 10 aa, synthetic construct
GFTFSSYVMS

SEQ ID NO: 2 - protein, 10 aa, synthetic construct
TINSNGGNTY

SEQ ID NO: 3 - protein, 14 aa, synthetic construct
DSLGLRRRDYAMDY

SEQ ID NO: 4 - protein, 10 aa, synthetic construct
GFTFSRYAMS

SEQ ID NO: 5 - protein, 9 aa, synthetic construct
SISRGGSTY

SEQ ID NO: 6 - protein, 10 aa, synthetic construct
YFGNYDAMDY

SEQ ID NO: 7 - protein, 10 aa, synthetic construct
GFAFSSYAMS

SEQ ID NO: 8 - protein, 9 aa, synthetic construct
SINRDVTTY

SEQ ID NO: 9 - protein, 14 aa, synthetic construct
GYYYGGGPYWHFDV

SEQ ID NO: 10 - protein, 10 aa, synthetic construct
GFTFSIYAMS

SEQ ID NO: 11 - protein, 9 aa, synthetic construct
SISGGGTAY

SEQ ID NO: 12 - protein, 14 aa, synthetic construct
GYYYGGSPYWHFDV

SEQ ID NO: 13 - protein, 9 aa, synthetic construct
SISTGGSPY

SEQ ID NO: 14 - protein, 14 aa, synthetic construct
GYYYNSSPHWYFAV

SEQ ID NO: 15 - protein, 10 aa, synthetic construct
GFTFSTYAMS

SEQ ID NO: 16 - protein, 9 aa, synthetic construct
SISTGASTY

SEQ ID NO: 17 - protein, 14 aa, synthetic construct
EETTTAALYYAMDY

SEQ ID NO: 18 - protein, 10 aa, synthetic construct
GFTFSSYAMS

SEQ ID NO: 19 - protein, 14 aa, synthetic construct
DYYYGSSLYYGMDY

SEQ ID NO: 20 - protein, 10 aa, synthetic construct
GFSFSNYAMS

SEQ ID NO: 21 - protein, 9 aa, synthetic construct
SINSGVTTY

SEQ ID NO: 22 - protein, 10 aa, synthetic construct
GFTFSNYIMS

SEQ ID NO: 23 - protein, 10 aa, synthetic construct
TINSGGTNTY

SEQ ID NO: 24 - protein, 10 aa, synthetic construct
YNGNYVWFAY

SEQ ID NO: 25 - protein, 9 aa, synthetic construct
SINRGGTTY

SEQ ID NO: 26 - protein, 14 aa, synthetic construct
DYYYGSSLYNGMDF

SEQ ID NO: 27 - protein, 14 aa, synthetic construct
DYYYGSNLYNGMDY

SEQ ID NO: 28 - protein, 11 aa, synthetic construct
VTSIDIDDDVN

SEQ ID NO: 29 - protein, 7 aa, synthetic construct
AGNTLRP

SEQ ID NO: 30 - protein, 9 aa, synthetic construct
LQSDNLPYT

SEQ ID NO: 31 - protein, 11 aa, synthetic construct
KASQDINNYVS

SEQ ID NO: 32 - protein, 7 aa, synthetic construct
RANRLVD

SEQ ID NO: 33 - protein, 9 aa, synthetic construct
LQFDEFPYT

SEQ ID NO: 34 - protein, 11 aa, synthetic construct
KASQDINSYLT

SEQ ID NO: 35 - protein, 11 aa, synthetic construct
KASQDINSYLS

SEQ ID NO: 36 - protein, 9 aa, synthetic construct
LQIDEFPYT

SEQ ID NO: 37 - protein, 9 aa, synthetic construct
LQYDEFPYT

SEQ ID NO: 38 - protein, 11 aa, synthetic construct
KASQDINNYLS

SEQ ID NO: 39 - protein, 10 aa, synthetic construct
SASSSVSFIY

SEQ ID NO: 40 - protein, 7 aa, synthetic construct
DTSNLAS

SEQ ID NO: 41 - protein, 9 aa, synthetic construct
QQWSNYHFT

SEQ ID NO: 42 - protein, 9 aa, synthetic construct
AISRGGSTY

SEQ ID NO: 43 - protein, 11 aa, synthetic construct
RASQDINNYVS

SEQ ID NO: 44 - protein, 11 aa, synthetic construct
RASQDINNYLS

SEQ ID NO: 45 - protein, 7 aa, synthetic construct
RANRLVD

SEQ ID NO: 46 - protein, 7 aa, synthetic construct
RANRLVS

SEQ ID NO: 47 - protein, 7 aa, synthetic construct
RANRLQS

SEQ ID NO: 48 - protein, 9 aa, synthetic construct
LQFDEFPYT

SEQ ID NO: 49 - protein, 11 aa, synthetic construct
QTSIDIDDDVN

SEQ ID NO: 50 - protein, 7 aa, synthetic construct
AGNTLET

SEQ ID NO: 51 - protein, 232 aa, synthetic construct
EPKSCDKTHTCPPCPAPELLGGPSVFLFPPKPKDTLMISRTPEVTCVVVDVSHEDPEVKFNWYVDGVEVHNAKTKPREEQYNSTYRVVSVLTVLHQDWLNGKEYKCKVSNKALPAPIEKTISKAKGQPREPQVYTLPPSRDELTKNQVSLTCLVKGFYPSDIAVEWESNGQPENNYKTTPPVLDSDGSFFLYSKLTVDKSRWQQGNVFSCSVMHEALHNHYTQKSLSLSPGK

SEQ ID NO: 52 - protein, 330 aa, synthetic construct [sequence omitted]

SEQ ID NO: 53 - protein, 107 aa, synthetic construct [sequence omitted]

SEQ ID NO: 54 - protein, 107 aa, synthetic construct
DIQMNQSPSSMYASLGERVTITCKASQDINNYVSWFQQKPGKSPKTLIYRANRLVDGVPSRFSGSGSGQDYSFTISSLEYEDMGIYYCLQFDEFPYTFGGGTKLEIK

SEQ ID NO: 55 - protein, 118 aa, synthetic construct
EVMLVESGGGLVKPGGSLKLSCAASGFTFSRYAMSWVRQTPEKRLEWVASISRGGSTYYPDSVKGRFTISRDNARNILYLQMSSLRSEDTAMYYCASYFGNYDAMDYWGQGTSVTVSS

SEQ ID NO: 56 - protein, 107 aa, synthetic construct
DIVLTQSPASLSMAIGEKVTIRCVTSIDIDDDVNWYQQKPGKPPKLLISAGNTLRPGVPSRFSSSGYGTDFVFTIENMLSEDVADYYCLQSDNLPYTFGGGTKLEIK

SEQ ID NO: 57 - protein, 123 aa, synthetic construct
DVKLVESGGGLVQPGGSLKLSCAASGFTFSSYVMSWVRQTPDKRLELVATINSNGGNTYYPDSVKGRFTISRDNAKNTLYLQMSSLKSEDTAMYYCARDSLGLRRRDYAMDYWGQGTSVTVSS

SEQ ID NO: 58 - protein, 107 aa, synthetic construct
DIQITQSPSSMYASLGERVTITCKASQDINSYLTWFQQKPGKSPKTLIYRANRLVDGVPSRFSGSGSGQDYSLTISSLEYEDMGIYYCLQFDEFPYTFGGGTKLEIK

SEQ ID NO: 59 - protein, 122 aa, synthetic construct
EVKLMESGGGLVKPGGSLKLSCAASGFAFSSYAMSWVRQTPDKRLEWVASINRDVTTYYPDSMKGRFTISRDNARNILYLQMSSLRSEDTAMYYCARGYYYGGGPYWHFDVWGAGTTVTVSS

SEQ ID NO: 60 - protein, 107 aa, synthetic construct
DIKMTQSPSSMYASLGERVTITCKASQDINSYLSWFQQKPGKSPKTLIYRANRLVDGVPSRFSGSGSGQDYSLTISSLEYEDIGIYYCLQIDEFPYTFGGGTKLEIK

SEQ ID NO: 61 - protein, 122 aa, synthetic construct
EVMLVESGGNLVKPGGSLKLSCAASGFTFSIYAMSWVRQTPEKRLEWVASISGGGTAYYPDSVKGRFTISRDNARNILYLQMSSLRSEDTAIYYCARGYYYGGSPYWHFDVWGAGTTVTVSS

SEQ ID NO: 62 - protein, 107 aa, synthetic construct
DIQMTQSPSSLSASLGERVTITCKASQDINSYLSWFQQKPGKSPKTLIYRANRLVDGVPSRFSGSGSGQDYSLTISSLEYEDMGIYYCLQYDEFPYTFGGGTKLEIK

SEQ ID NO: 63 - protein, 122 aa, synthetic construct
EVQLVESGGGLVQPKGSLKLSCAASGFTFSRYAMSWVRQTPEKRLEWVASISTGGSPYYPDSVKGRFTISRDNARNILYLQMSSLKSEDTAMYYCARGYYYNSSPHWYFAVWGAGTSVTVSS

SEQ ID NO: 64 - protein, 107 aa, synthetic construct
DIKITQSPSSMYASLGERVTITCKASQDINNYLSWFQQKPGKSPKTLIYRANRLVDGVPSRFSGSGSGQDYSLTISSLEYEDMGIYYCLQFDEFPYTFGGGTKLEIK

SEQ ID NO: 65 - protein, 122 aa, synthetic construct
EVKLVESGGGLVKPGGSLKLSCAASGFTFSTYAMSWVRQTPEKRLEWVASISTGASTYYPDSVKGRFTISRDNARNILYLQMSSLRSEDTAMYYCAREETTTAALYYAMDYWGQGTSVTVSS

SEQ ID NO: 66 - protein, 107 aa, synthetic construct
DIQMTQSPSSMHASLGERVTITCKASQDINNYVSWFQQKPGKSPKTLIYRANRLVDGVPSRFSGSGSGQDYSFTISSLEYEDMGIYYCLQFDEFPYTFGGGTKLEIK

SEQ ID NO: 67 - protein, 122 aa, synthetic construct
EVMLVESGGGLVRPGGSLKLSCAASGFTFSSYAMSWVRQTPDKRLEWVASINRDVTTYYPDSVKGRFTISRDNARNILYLQMSSLRSEDTAMYYCARDYYYGSSLYYGMDYWGQGTSVTVSS

SEQ ID NO: 68 - protein, 122 aa, synthetic construct
EVKLVESGGGLVKPGGSLKLSCAASGFSFSNYAMSWVRQTPEKRLEWVASINSGVTTYYPDSVKGRFTVSRDNARNILYLHMTGLRSEDTAIYYCSRGYYYGGSPYWHFDVWGAGTTVTVSS

SEQ ID NO: 69 - protein, 106 aa, synthetic construct
DIVLTQSPAIMSASPGEKVTMTCSASSSVSFIYWYQQKPGSSPRLLIYDTSNLASGVPVRFSGSGSGTSYSLTISRMEAEDAATYYCQQWSNYHFTFGSGTKLEIK

SEQ ID NO: 70 - protein, 119 aa, synthetic construct
EVMLVESGGGLVKPGGSLKLSCAASGFTFSNYIMSWVRQTPEKRLEWVATINSGGTNTYYPDSVKGRFTISRDNAKNSLYLQMNSLRSEDTALYYCTRYNGNYVWFAYWGQGTLVTVSA

SEQ ID NO: 71 - protein, 107 aa, synthetic construct
DIQMTQSPSSMYASLGERVTITCKASQDINSYLSWFQQKPGKSPKTLIYRANRLVDGVPSRFSGSGSGQDYSLTISSLESEDMGIYYCLQFDEFPYTFGGGTKLEIK

SEQ ID NO: 72 - protein, 122 aa, synthetic construct
EVMLVESGGGLVKPGGSLKLSCAASGFTFSRYAMSWVRQTPEKRLEWVASINRGGTTYYPDSVKGRFTISRDNARDILYLQMSSLRSEDTAIYYCARDYYYGSSLYNGMDFWGQGTSVIVSS

SEQ ID NO: 73 - protein, 107 aa, synthetic construct
DIKITQSPSSMYASLGERVTITCKASQDINSYLSWFQQKPGKSPKTLIYRANRLVDGVPSRFSGSGSGQDYSLTISSLEYEDMGIYYCLQFDEFPYTFGGGTKLEIK

SEQ ID NO: 74 - protein, 122 aa, synthetic construct
EVMLVESGGGLVRPGGSLKLSCAASGFTFSSYAMSWVRQSPEKRLEWVASINRGGTTYYPDSVKGRFTISRDNARDILYLQMSSLRSEDTAIYYCARDYYYGSNLYNGMDYWGQGTSVIVSS

SEQ ID NO: 75 - protein, 118 aa, synthetic construct
EVQLVESGGGLVQPGGSLRLSCAASGFTFSRYAMSWVRQTPGKRLEWVASISRGGSTYYPDSVKGRFTISRDNAKNTLYLQMSSLRAEDTAMYYCASYFGNYDAMDYWGQGTTVTVSS

SEQ ID NO: 76 - protein, 118 aa, synthetic construct
EVQLVESGGGLVQPGGSLRLSCAASGFTFSRYAMSWVRQAPGKGLEWVASISRGGSTYYADSVKGRFTISRDNAKNTLYLQMSSLRAEDTAVYYCASYFGNYDAMDYWGQGTTVTVSS

SEQ ID NO: 77 - protein, 118 aa, synthetic construct
EVQLVESGGGLVQPGGSLRLSCAASGFTFSRYAMSWVRQAPGKGLEWVASISRGGSTYYADSVKGRFTISRDNSKNTLYLQMNSLRAEDTAVYYCASYFGNYDAMDYWGQGTTVTVSS

SEQ ID NO: 78 - protein, 118 aa, synthetic construct
EVQLVESGGGLVQPGGSLRLSCAASGFTFSRYAMSWVRQAPGKGLEWVSAISRGGSTYYADSVKGRFTISRDNSKNTLYLQMNSLRAEDTAVYYCASYFGNYDAMDYWGQGTTVTVSS

SEQ ID NO: 79 - protein, 107 aa, synthetic construct
DIQMTQSPSSLSASVGDRVTITCKASQDINNYVSWFQQKPGKAPKTLIYRANRLVDGVPSRFSGSGSGQDYTFTISSLQPEDFATYYCLQFDEFPYTFGGGTKLEIK

SEQ ID NO: 80 - protein, 107 aa, synthetic construct
DIQMTQSPSSLSASVGDRVTITCKASQDINNYVSWFQQKPGKAPKSLIYRANRLVDGVPSRFSGSGSGTDYTFTISSLQPEDFATYYCLQFDEFPYTFGGGTKLEIK

SEQ ID NO: 81 - protein, 107 aa, synthetic construct
DIQMTQSPSSLSASVGDRVTITCRASQDINNYVSWFQQKPGKAPKSLIYRANRLVSGVPSRFSGSGSGTDFTFTISSLQPEDFATYYCLQFDEFPYTFGGGTKLEIK

SEQ ID NO: 82 - protein, 107 aa, synthetic construct
DIQMTQSPSSLSASVGDRVTITCRASQDINNYLSWFQQKPGKAPKSLIYRANRLQSGVPSRFSGSGSGTDFTLTISSLQPEDFATYYCLQFDEFPYTFGGGTKLEIK

SEQ ID NO: 83 - protein, 123 aa, synthetic construct
EVQLVESGGGLVQPGGSLRLSCAASGFTFSSYVMSWVRQTPGKRLELVATINSNGGNTYYPDSVKGRFTISRDNAKNTLYLQMSSLRAEDTAMYYCARDSLGLRRRDYAMDYWGQGTTVTVSS

SEQ ID NO: 84 - protein, 123 aa, synthetic construct
EVQLVESGGGLVQPGGSLRLSCAASGFTFSSYVMSWVRQAPGKGLELVATINSNGGNTYYPDSVKGRFTISRDNAKNTLYLQMGSLRAEDTAMYYCARDSLGLRRRDYAMDYWGQGTTVTVSS

SEQ ID NO: 85 - protein, 123 aa, synthetic construct
EVQLVESGGGLVQPGGSLRLSCAASGFTFSSYVMSWVRQAPGKGLEYVATINSNGGNTYYADSVKGRFTISRDNSKNTLYLQMGSLRAEDTAMYYCARDSLGLRRRDYAMDYWGQGTTVTVSS

SEQ ID NO: 86 - protein, 107 aa, synthetic construct
DIQLTQSPSSLSASVGDRVTIRCVTSIDIDDDVNWYQQKPGKAPKLLISAGNTLRPGVPSRFSSSGYGTDFTFTISSMQPEDIATYYCLQSDNLPYTFGGGTKLEIK

SEQ ID NO: 87 - protein, 107 aa, synthetic construct
DIQLTQSPSSLSASVGDRVTIRCVTSIDIDDDVNWYQQKPGKAPKLLISAGNTLRPGVPSRFSGSGSGTDFTFTISSLQPEDIATYYCLQSDNLPYTFGGGTKLEIK

SEQ ID NO: 88 - protein, 107 aa, synthetic construct
DIQMTQSPSSLSASVGDRVTITCVTSIDIDDDVNWYQQKPGKAPKLLISAGNTLRPGVPSRFSGSGSGTDFTFTISSLQPEDIATYYCLQSDNLPYTFGGGTKLEIK

SEQ ID NO: 89 - protein, 107 aa, synthetic construct
DIQMTQSPSSLSASVGDRVTITCQTSIDIDDDVNWYQQKPGKAPKLLISAGNTLETGVPSRFSGSGSGTDFTFTISSLQPEDIATYYCLQSDNLPYTFGGGTKLEIK

SEQ ID NO: 90 - protein, 214 aa, synthetic construct
DIQMNQSPSSMYASLGERVTITCKASQDINNYVSWFQQKPGKSPKTLIYRANRLVDGVPSRFSGSGSGQDYSFTISSLEYEDMGIYYCLQFDEFPYTFGGGTKLEIKRTVAAPSVFIFPPSDEQLKSGTASVVCLLNNFYPREAKVQWKVDNALQSGNSQESVTEQDSKDSTYSLSSTLTLSKADYEKHKVYACEVTHQGLSSPVTKSFNRGEC

SEQ ID NO: 91 - protein, 448 aa, synthetic construct
EVMLVESGGGLVKPGGSLKLSCAASGFTFSRYAMSWVRQTPEKRLEWVASISRGGSTYYPDSVKGRFTISRDNARNILYLQMSSLRSEDTAMYYCASYFGNYDAMDYWGQGTSVTVSSASTKGPSVFPLAPSSKSTSGGTAALGCLVKDYFPEPVTVSWNSGALTSGVHTFPAVLQSSGLYSLSSVVTVPSSSLGTQTYICNVNHKPSNTKVDKKVEPKSCDKTHTCPPCPAPELLGGPSVFLFPPKPKDTLMISRTPEVTCVVVDVSHEDPEVKFNWYVDGVEVHNAKTKPREEQYNSTYRVVSVLTVLHQDWLNGKEYKCKVSNKALPAPIEKTISKAKGQPREPQVYTLPPSRDELTKNQVSLTCLVKGFYPSDIAVEWESNGQPENNYKTTPPVLDSDGSFFLYSKLTVDKSRWQQGNVFSCSVMHEALHNHYTQKSLSLSPGK

SEQ ID NO: 92 - protein, 214 aa, synthetic construct
DIVLTQSPASLSMAIGEKVTIRCVTSIDIDDDVNWYQQKPGKPPKLLISAGNTLRPGVPSRFSSSGYGTDFVFTIENMLSEDVADYYCLQSDNLPYTFGGGTKLEIKRTVAAPSVFIFPPSDEQLKSGTASVVCLLNNFYPREAKVQWKVDNALQSGNSQESVTEQDSKDSTYSLSSTLTLSKADYEKHKVYACEVTHQGLSSPVTKSFNRGEC

SEQ ID NO: 93 - protein, 453 aa, synthetic construct
DVKLVESGGGLVQPGGSLKLSCAASGFTFSSYVMSWVRQTPDKRLELVATINSNGGNTYYPDSVKGRFTISRDNAKNTLYLQMSSLKSEDTAMYYCARDSLGLRRRDYAMDYWGQGTSVTVSSASTKGPSVFPLAPSSKSTSGGTAALGCLVKDYFPEPVTVSWNSGALTSGVHTFPAVLQSSGLYSLSSVVTVPSSSLGTQTYICNVNHKPSNTKVDKKVEPKSCDKTHTCPPCPAPELLGGPSVFLFPPKPKDTLMISRTPEVTCVVVDVSHEDPEVKFNWYVDGVEVHNAKTKPREEQYNSTYRVVSVLTVLHQDWLNGKEYKCKVSNKALPAPIEKTISKAKGQPREPQVYTLPPSRDELTKNQVSLTCLVKGFYPSDIAVEWESNGQPENNYKTTPPVLDSDGSFFLYSKLTVDKSRWQQGNVFSCSVMHEALHNHYTQKSLSLSPGK

SEQ ID NO: 94 - protein, 214 aa, synthetic construct
DIQITQSPSSMYASLGERVTITCKASQDINSYLTWFQQKPGKSPKTLIYRANRLVDGVPSRFSGSGSGQDYSLTISSLEYEDMGIYYCLQFDEFPYTFGGGTKLEIKRTVAAPSVFIFPPSDEQLKSGTASVVCLLNNFYPREAKVQWKVDNALQSGNSQESVTEQDSKDSTYSLSSTLTLSKADYEKHKVYACEVTHQGLSSPVTKSFNRGEC

SEQ ID NO: 95 - protein, 452 aa, synthetic construct
EVKLMESGGGLVKPGGSLKLSCAASGFAFSSYAMSWVRQTPDKRLEWVASINRDVTTYYPDSMKGRFTISRDNARNILYLQMSSLRSEDTAMYYCARGYYYGGGPYWHFDVWGAGTTVTVSSASTKGPSVFPLAPSSKSTSGGTAALGCLVKDYFPEPVTVSWNSGALTSGVHTFPAVLQSSGLYSLSSVVTVPSSSLGTQTYICNVNHKPSNTKVDKKVEPKSCDKTHTCPPCPAPELLGGPSVFLFPPKPKDTLMISRTPEVTCVVVDVSHEDPEVKFNWYVDGVEVHNAKTKPREEQYNSTYRVVSVLTVLHQDWLNGKEYKCKVSNKALPAPIEKTISKAKGQPREPQVYTLPPSRDELTKNQVSLTCLVKGFYPSDIAVEWESNGQPENNYKTTPPVLDSDGSFFLYSKLTVDKSRWQQGNVFSCSVMHEALHNHYTQKSLSLSPGK

SEQ ID NO: 96 - protein, 214 aa, synthetic construct
DIKMTQSPSSMYASLGERVTITCKASQDINSYLSWFQQKPGKSPKTLIYRANRLVDGVPSRFSGSGSGQDYSLTISSLEYEDIGIYYCLQIDEFPYTFGGGTKLEIKRTVAAPSVFIFPPSDEQLKSGTASVVCLLNNFYPREAKVQWKVDNALQSGNSQESVTEQDSKDSTYSLSSTLTLSKADYEKHKVYACEVTHQGLSSPVTKSFNRGEC

SEQ ID NO: 97 - protein, 452 aa, synthetic construct
EVMLVESGGNLVKPGGSLKLSCAASGFTFSIYAMSWVRQTPEKRLEWVASISGGGTAYYPDSVKGRFTISRDNARNILYLQMSSLRSEDTAIYYCARGYYYGGSPYWHFDVWGAGTTVTVSSASTKGPSVFPLAPSSKSTSGGTAALGCLVKDYFPEPVTVSWNSGALTSGVHTFPAVLQSSGLYSLSSVVTVPSSSLGTQTYICNVNHKPSNTKVDKKVEPKSCDKTHTCPPCPAPELLGGPSVFLFPPKPKDTLMISRTPEVTCVVVDVSHEDPEVKFNWYVDGVEVHNAKTKPREEQYNSTYRVVSVLTVLHQDWLNGKEYKCKVSNKALPAPIEKTISKAKGQPREPQVYTLPPSRDELTKNQVSLTCLVKGFYPSDIAVEWESNGQPENNYKTTPPVLDSDGSFFLYSKLTVDKSRWQQGNVFSCSVMHEALHNHYTQKSLSLSPGK

SEQ ID NO: 98 - protein, 214 aa, synthetic construct
DIQMTQSPSSLSASLGERVTITCKASQDINSYLSWFQQKPGKSPKTLIYRANRLVDGVPSRFSGSGSGQDYSLTISSLEYEDMGIYYCLQYDEFPYTFGGGTKLEIKRTVAAPSVFIFPPSDEQLKSGTASVVCLLNNFYPREAKVQWKVDNALQSGNSQESVTEQDSKDSTYSLSSTLTLSKADYEKHKVYACEVTHQGLSSPVTKSFNRGEC

SEQ ID NO: 99 - protein, 452 aa, synthetic construct
EVQLVESGGGLVQPKGSLKLSCAASGFTFSRYAMSWVRQTPEKRLEWVASISTGGSPYYPDSVKGRFTISRDNARNILYLQMSSLKSEDTAMYYCARGYYYNSSPHWYFAVWGAGTSVTVSSASTKGPSVFPLAPSSKSTSGGTAALGCLVKDYFPEPVTVSWNSGALTSGVHTFPAVLQSSGLYSLSSVVTVPSSSLGTQTYICNVNHKPSNTKVDKKVEPKSCDKTHTCPPCPAPELLGGPSVFLFPPKPKDTLMISRTPEVTCVVVDVSHEDPEVKFNWYVDGVEVHNAKTKPREEQYNSTYRVVSVLTVLHQDWLNGKEYKCKVSNKALPAPIEKTISKAKGQPREPQVYTLPPSRDELTKNQVSLTCLVKGFYPSDIAVEWESNGQPENNYKTTPPVLDSDGSFFLYSKLTVDKSRWQQGNVFSCSVMHEALHNHYTQKSLSLSPGK

SEQ ID NO: 100 - protein, 214 aa, synthetic construct
DIKITQSPSSMYASLGERVTITCKASQDINNYLSWFQQKPGKSPKTLIYRANRLVDGVPSRFSGSGSGQDYSLTISSLEYEDMGIYYCLQFDEFPYTFGGGTKLEIKRTVAAPSVFIFPPSDEQLKSGTASVVCLLNNFYPREAKVQWKVDNALQSGNSQESVTEQDSKDSTYSLSSTLTLSKADYEKHKVYACEVTHQGLSSPVTKSFNRGEC

SEQ ID NO: 101 - protein, 452 aa, synthetic construct
EVKLVESGGGLVKPGGSLKLSCAASGFTFSTYAMSWVRQTPEKRLEWVASISTGASTYYPDSVKGRFTISRDNARNILYLQMSSLRSEDTAMYYCAREETTTAALYYAMDYWGQGTSVTVSSASTKGPSVFPLAPSSKSTSGGTAALGCLVKDYFPEPVTVSWNSGALTSGVHTFPAVLQSSGLYSLSSVVTVPSSSLGTQTYICNVNHKPSNTKVDKKVEPKSCDKTHTCPPCPAPELLGGPSVFLFPPKPKDTLMISRTPEVTCVVVDVSHEDPEVKFNWYVDGVEVHNAKTKPREEQYNSTYRVVSVLTVLHQDWLNGKEYKCKVSNKALPAPIEKTISKAKGQPREPQVYTLPPSRDELTKNQVSLTCLVKGFYPSDIAVEWESNGQPENNYKTTPPVLDSDGSFFLYSKLTVDKSRWQQGNVFSCSVMHEALHNHYTQKSLSLSPGK

SEQ ID NO: 102 - protein, 214 aa, synthetic construct
DIQMTQSPSSMHASLGERVTITCKASQDINNYVSWFQQKPGKSPKTLIYRANRLVDGVPSRFSGSGSGQDYSFTISSLEYEDMGIYYCLQFDEFPYTFGGGTKLEIKRTVAAPSVFIFPPSDEQLKSGTASVVCLLNNFYPREAKVQWKVDNALQSGNSQESVTEQDSKDSTYSLSSTLTLSKADYEKHKVYACEVTHQGLSSPVTKSFNRGEC

SEQ ID NO: 103 - protein, 452 aa, synthetic construct
EVMLVESGGGLVRPGGSLKLSCAASGFTFSSYAMSWVRQTPDKRLEWVASINRDVTTYYPDSVKGRFTISRDNARNILYLQMSSLRSEDTAMYYCARDYYYGSSLYYGMDYWGQGTSVTVSSASTKGPSVFPLAPSSKSTSGGTAALGCLVKDYFPEPVTVSWNSGALTSGVHTFPAVLQSSGLYSLSSVVTVPSSSLGTQTYICNVNHKPSNTKVDKKVEPKSCDKTHTCPPCPAPELLGGPSVFLFPPKPKDTLMISRTPEVTCVVVDVSHEDPEVKFNWYVDGVEVHNAKTKPREEQYNSTYRVVSVLTVLHQDWLNGKEYKCKVSNKALPAPIEKTISKAKGQPREPQVYTLPPSRDELTKNQVSLTCLVKGFYPSDIAVEWESNGQPENNYKTTPPVLDSDGSFFLYSKLTVDKSRWQQGNVFSCSVMHEALHNHYTQKSLSLSPGK

SEQ ID NO: 104 - protein, 452 aa, synthetic construct
EVKLVESGGGLVKPGGSLKLSCAASGFSFSNYAMSWVRQTPEKRLEWVASINSGVTTYYPDSVKGRFTVSRDNARNILYLHMTGLRSEDTAIYYCSRGYYYGGSPYWHFDVWGAGTTVTVSSASTKGPSVFPLAPSSKSTSGGTAALGCLVKDYFPEPVTVSWNSGALTSGVHTFPAVLQSSGLYSLSSVVTVPSSSLGTQTYICNVNHKPSNTKVDKKVEPKSCDKTHTCPPCPAPELLGGPSVFLFPPKPKDTLMISRTPEVTCVVVDVSHEDPEVKFNWYVDGVEVHNAKTKPREEQYNSTYRVVSVLTVLHQDWLNGKEYKCKVSNKALPAPIEKTISKAKGQPREPQVYTLPPSRDELTKNQVSLTCLVKGFYPSDIAVEWESNGQPENNYKTTPPVLDSDGSFFLYSKLTVDKSRWQQGNVFSCSVMHEALHNHYTQKSLSLSPGK

SEQ ID NO: 105 - protein, 213 aa, synthetic construct
DIVLTQSPAIMSASPGEKVTMTCSASSSVSFIYWYQQKPGSSPRLLIYDTSNLASGVPVRFSGSGSGTSYSLTISRMEAEDAATYYCQQWSNYHFTFGSGTKLEIKRTVAAPSVFIFPPSDEQLKSGTASVVCLLNNFYPREAKVQWKVDNALQSGNSQESVTEQDSKDSTYSLSSTLTLSKADYEKHKVYACEVTHQGLSSPVTKSFNRGEC

SEQ ID NO: 106 - protein, 449 aa, synthetic construct
EVMLVESGGGLVKPGGSLKLSCAASGFTFSNYIMSWVRQTPEKRLEWVATINSGGTNTYYPDSVKGRFTISRDNAKNSLYLQMNSLRSEDTALYYCTRYNGNYVWFAYWGQGTLVTVSAASTKGPSVFPLAPSSKSTSGGTAALGCLVKDYFPEPVTVSWNSGALTSGVHTFPAVLQSSGLYSLSSVVTVPSSSLGTQTYICNVNHKPSNTKVDKKVEPKSCDKTHTCPPCPAPELLGGPSVFLFPPKPKDTLMISRTPEVTCVVVDVSHEDPEVKFNWYVDGVEVHNAKTKPREEQYNSTYRVVSVLTVLHQDWLNGKEYKCKVSNKALPAPIEKTISKAKGQPREPQVYTLPPSRDELTKNQVSLTCLVKGFYPSDIAVEWESNGQPENNYKTTPPVLDSDGSFFLYSKLTVDKSRWQQGNVFSCSVMHEALHNHYTQKSLSLSPGK

SEQ ID NO: 107 - protein, 214 aa, synthetic construct
DIQMTQSPSSMYASLGERVTITCKASQDINSYLSWFQQKPGKSPKTLIYRANRLVDGVPSRFSGSGSGQDYSLTISSLESEDMGIYYCLQFDEFPYTFGGGTKLEIKRTVAAPSVFIFPPSDEQLKSGTASVVCLLNNFYPREAKVQWKVDNALQSGNSQESVTEQDSKDSTYSLSSTLTLSKADYEKHKVYACEVTHQGLSSPVTKSFNRGEC

SEQ ID NO: 108 - protein, 452 aa, synthetic construct
EVMLVESGGGLVKPGGSLKLSCAASGFTFSRYAMSWVRQTPEKRLEWVASINRGGTTYYPDSVKGRFTISRDNARDILYLQMSSLRSEDTAIYYCARDYYYGSSLYNGMDFWGQGTSVIVSSASTKGPSVFPLAPSSKSTSGGTAALGCLVKDYFPEPVTVSWNSGALTSGVHTFPAVLQSSGLYSLSSVVTVPSSSLGTQTYICNVNHKPSNTKVDKKVEPKSCDKTHTCPPCPAPELLGGPSVFLFPPKPKDTLMISRTPEVTCVVVDVSHEDPEVKFNWYVDGVEVHNAKTKPREEQYNSTYRVVSVLTVLHQDWLNGKEYKCKVSNKALPAPIEKTISKAKGQPREPQVYTLPPSRDELTKNQVSLTCLVKGFYPSDIAVEWESNGQPENNYKTTPPVLDSDGSFFLYSKLTVDKSRWQQGNVFSCSVMHEALHNHYTQKSLSLSPGK

SEQ ID NO: 109 - protein, 214 aa, synthetic construct
DIKITQSPSSMYASLGERVTITCKASQDINSYLSWFQQKPGKSPKTLIYRANRLVDGVPSRFSGSGSGQDYSLTISSLEYEDMGIYYCLQFDEFPYTFGGGTKLEIKRTVAAPSVFIFPPSDEQLKSGTASVVCLLNNFYPREAKVQWKVDNALQSGNSQESVTEQDSKDSTYSLSSTLTLSKADYEKHKVYACEVTHQGLSSPVTKSFNRGEC

SEQ ID NO: 110 - protein, 452 aa, synthetic construct
EVMLVESGGGLVRPGGSLKLSCAASGFTFSSYAMSWVRQSPEKRLEWVASINRGGTTYYPDSVKGRFTISRDNARDILYLQMSSLRSEDTAIYYCARDYYYGSNLYNGMDYWGQGTSVIVSSASTKGPSVFPLAPSSKSTSGGTAALGCLVKDYFPEPVTVSWNSGALTSGVHTFPAVLQSSGLYSLSSVVTVPSSSLGTQTYICNVNHKPSNTKVDKKVEPKSCDKTHTCPPCPAPELLGGPSVFLFPPKPKDTLMISRTPEVTCVVVDVSHEDPEVKFNWYVDGVEVHNAKTKPREEQYNSTYRVVSVLTVLHQDWLNGKEYKCKVSNKALPAPIEKTISKAKGQPREPQVYTLPPSRDELTKNQVSLTCLVKGFYPSDIAVEWESNGQPENNYKTTPPVLDSDGSFFLYSKLTVDKSRWQQGNVFSCSVMHEALHNHYTQKSLSLSPGK

SEQ ID NO: 111 - protein, 448 aa, synthetic construct
EVQLVESGGGLVQPGGSLRLSCAASGFTFSRYAMSWVRQTPGKRLEWVASISRGGSTYYPDSVKGRFTISRDNAKNTLYLQMSSLRAEDTAMYYCASYFGNYDAMDYWGQGTTVTVSSASTKGPSVFPLAPSSKSTSGGTAALGCLVKDYFPEPVTVSWNSGALTSGVHTFPAVLQSSGLYSLSSVVTVPSSSLGTQTYICNVNHKPSNTKVDKKVEPKSCDKTHTCPPCPAPELLGGPSVFLFPPKPKDTLMISRTPEVTCVVVDVSHEDPEVKFNWYVDGVEVHNAKTKPREEQYNSTYRVVSVLTVLHQDWLNGKEYKCKVSNKALPAPIEKTISKAKGQPREPQVYTLPPSRDELTKNQVSLTCLVKGFYPSDIAVEWESNGQPENNYKTTPPVLDSDGSFFLYSKLTVDKSRWQQGNVFSCSVMHEALHNHYTQKSLSLSPGK

SEQ ID NO: 112 - protein, 448 aa, synthetic construct
EVQLVESGGGLVQPGGSLRLSCAASGFTFSRYAMSWVRQAPGKGLEWVASISRGGSTYYADSVKGRFTISRDNAKNTLYLQMSSLRAEDTAVYYCASYFGNYDAMDYWGQGTTVTVSSASTKGPSVFPLAPSSKSTSGGTAALGCLVKDYFPEPVTVSWNSGALTSGVHTFPAVLQSSGLYSLSSVVTVPSSSLGTQTYICNVNHKPSNTKVDKKVEPKSCDKTHTCPPCPAPELLGGPSVFLFPPKPKDTLMISRTPEVTCVVVDVSHEDPEVKFNWYVDGVEVHNAKTKPREEQYNSTYRVVSVLTVLHQDWLNGKEYKCKVSNKALPAPIEKTISKAKGQPREPQVYTLPPSRDELTKNQVSLTCLVKGFYPSDIAVEWESNGQPENNYKTTPPVLDSDGSFFLYSKLTVDKSRWQQGNVFSCSVMHEALHNHYTQKSLSLSPGK

SEQ ID NO: 113 - protein, 448 aa, synthetic construct
EVQLVESGGGLVQPGGSLRLSCAASGFTFSRYAMSWVRQAPGKGLEWVASISRGGSTYYADSVKGRFTISRDNSKNTLYLQMNSLRAEDTAVYYCASYFGNYDAMDYWGQGTTVTVSSASTKGPSVFPLAPSSKSTSGGTAALGCLVKDYFPEPVTVSWNSGALTSGVHTFPAVLQSSGLYSLSSVVTVPSSSLGTQTYICNVNHKPSNTKVDKKVEPKSCDKTHTCPPCPAPELLGGPSVFLFPPKPKDTLMISRTPEVTCVVVDVSHEDPEVKFNWYVDGVEVHNAKTKPREEQYNSTYRVVSVLTVLHQDWLNGKEYKCKVSNKALPAPIEKTISKAKGQPREPQVYTLPPSRDELTKNQVSLTCLVKGFYPSDIAVEWESNGQPENNYKTTPPVLDSDGSFFLYSKLTVDKSRWQQGNVFSCSVMHEALHNHYTQKSLSLSPGK

SEQ ID NO: 114 - protein, 448 aa, synthetic construct
EVQLVESGGGLVQPGGSLRLSCAASGFTFSRYAMSWVRQAPGKGLEWVSAISRGGSTYYADSVKGRFTISRDNSKNTLYLQMNSLRAEDTAVYYCASYFGNYDAMDYWGQGTTVTVSSASTKGPSVFPLAPSSKSTSGGTAALGCLVKDYFPEPVTVSWNSGALTSGVHTFPAVLQSSGLYSLSSVVTVPSSSLGTQTYICNVNHKPSNTKVDKKVEPKSCDKTHTCPPCPAPELLGGPSVFLFPPKPKDTLMISRTPEVTCVVVDVSHEDPEVKFNWYVDGVEVHNAKTKPREEQYNSTYRVVSVLTVLHQDWLNGKEYKCKVSNKALPAPIEKTISKAKGQPREPQVYTLPPSRDELTKNQVSLTCLVKGFYPSDIAVEWESNGQPENNYKTTPPVLDSDGSFFLYSKLTVDKSRWQQGNVFSCSVMHEALHNHYTQKSLSLSPGK

SEQ ID NO: 115 - protein, 214 aa, synthetic construct
DIQMTQSPSSLSASVGDRVTITCKASQDINNYVSWFQQKPGKAPKTLIYRANRLVDGVPSRFSGSGSGQDYTFTISSLQPEDFATYYCLQFDEFPYTFGGGTKLEIKRTVAAPSVFIFPPSDEQLKSGTASVVCLLNNFYPREAKVQWKVDNALQSGNSQESVTEQDSKDSTYSLSSTLTLSKADYEKHKVYACEVTHQGLSSPVTKSFNRGEC

SEQ ID NO: 116 - protein, 214 aa, synthetic construct
DIQMTQSPSSLSASVGDRVTITCKASQDINNYVSWFQQKPGKAPKSLIYRANRLVDGVPSRFSGSGSGTDYTFTISSLQPEDFATYYCLQFDEFPYTFGGGTKLEIKRTVAAPSVFIFPPSDEQLKSGTASVVCLLNNFYPREAKVQWKVDNALQSGNSQESVTEQDSKDSTYSLSSTLTLSKADYEKHKVYACEVTHQGLSSPVTKSFNRGEC

SEQ ID NO: 117 - protein, 214 aa, synthetic construct
DIQMTQSPSSLSASVGDRVTITCRASQDINNYVSWFQQKPGKAPKSLIYRANRLVSGVPSRFSGSGSGTDFTFTISSLQPEDFATYYCLQFDEFPYTFGGGTKLEIKRTVAAPSVFIFPPSDEQLKSGTASVVCLLNNFYPREAKVQWKVDNALQSGNSQESVTEQDSKDSTYSLSSTLTLSKADYEKHKVYACEVTHQGLSSPVTKSFNRGEC

SEQ ID NO: 118 - protein, 214 aa, synthetic construct
DIQMTQSPSSLSASVGDRVTITCRASQDINNYLSWFQQKPGKAPKSLIYRANRLQSGVPSRFSGSGSGTDFTLTISSLQPEDFATYYCLQFDEFPYTFGGGTKLEIKRTVAAPSVFIFPPSDEQLKSGTASVVCLLNNFYPREAKVQWKVDNALQSGNSQESVTEQDSKDSTYSLSSTLTLSKADYEKHKVYACEVTHQGLSSPVTKSFNRGEC

SEQ ID NO: 119 - protein, 453 aa, synthetic construct
EVQLVESGGGLVQPGGSLRLSCAASGFTFSSYVMSWVRQTPGKRLELVATINSNGGNTYYPDSVKGRFTISRDNAKNTLYLQMSSLRAEDTAMYYCARDSLGLRRRDYAMDYWGQGTTVTVSSASTKGPSVFPLAPSSKSTSGGTAALGCLVKDYFPEPVTVSWNSGALTSGVHTFPAVLQSSGLYSLSSVVTVPSSSLGTQTYICNVNHKPSNTKVDKKVEPKSCDKTHTCPPCPAPELLGGPSVFLFPPKPKDTLMISRTPEVTCVVVDVSHEDPEVKFNWYVDGVEVHNAKTKPREEQYNSTYRVVSVLTVLHQDWLNGKEYKCKVSNKALPAPIEKTISKAKGQPREPQVYTLPPSRDELTKNQVSLTCLVKGFYPSDIAVEWESNGQPENNYKTTPPVLDSDGSFFLYSKLTVDKSRWQQGNVFSCSVMHEALHNHYTQKSLSLSPGK

SEQ ID NO: 120 - protein, 453 aa, synthetic construct
EVQLVESGGGLVQPGGSLRLSCAASGFTFSSYVMSWVRQAPGKGLELVATINSNGGNTYYPDSVKGRFTISRDNAKNTLYLQMGSLRAEDTAMYYCARDSLGLRRRDYAMDYWGQGTTVTVSSASTKGPSVFPLAPSSKSTSGGTAALGCLVKDYFPEPVTVSWNSGALTSGVHTFPAVLQSSGLYSLSSVVTVPSSSLGTQTYICNVNHKPSNTKVDKKVEPKSCDKTHTCPPCPAPELLGGPSVFLFPPKPKDTLMISRTPEVTCVVVDVSHEDPEVKFNWYVDGVEVHNAKTKPREEQYNSTYRVVSVLTVLHQDWLNGKEYKCKVSNKALPAPIEKTISKAKGQPREPQVYTLPPSRDELTKNQVSLTCLVKGFYPSDIAVEWESNGQPENNYKTTPPVLDSDGSFFLYSKLTVDKSRWQQGNVFSCSVMHEALHNHYTQKSLSLSPGK

SEQ ID NO: 121 - protein, 453 aa, synthetic construct
EVQLVESGGGLVQPGGSLRLSCAASGFTFSSYVMSWVRQAPGKGLEYVATINSNGGNTYYADSVKGRFTISRDNSKNTLYLQMGSLRAEDTAMYYCARDSLGLRRRDYAMDYWGQGTTVTVSSASTKGPSVFPLAPSSKSTSGGTAALGCLVKDYFPEPVTVSWNSGALTSGVHTFPAVLQSSGLYSLSSVVTVPSSSLGTQTYICNVNHKPSNTKVDKKVEPKSCDKTHTCPPCPAPELLGGPSVFLFPPKPKDTLMISRTPEVTCVVVDVSHEDPEVKFNWYVDGVEVHNAKTKPREEQYNSTYRVVSVLTVLHQDWLNGKEYKCKVSNKALPAPIEKTISKAKGQPREPQVYTLPPSRDELTKNQVSLTCLVKGFYPSDIAVEWESNGQPENNYKTTPPVLDSDGSFFLYSKLTVDKSRWQQGNVFSCSVMHEALHNHYTQKSLSLSPGK

SEQ ID NO: 122 - protein, 214 aa, synthetic construct
DIQLTQSPSSLSASVGDRVTIRCVTSIDIDDDVNWYQQKPGKAPKLLISAGNTLRPGVPSRFSSSGYGTDFTFTISSMQPEDIATYYCLQSDNLPYTFGGGTKLEIKRTVAAPSVFIFPPSDEQLKSGTASVVCLLNNFYPREAKVQWKVDNALQSGNSQESVTEQDSKDSTYSLSSTLTLSKADYEKHKVYACEVTHQGLSSPVTKSFNRGEC

SEQ ID NO: 123 - protein, 214 aa, synthetic construct
DIQLTQSPSSLSASVGDRVTIRCVTSIDIDDDVNWYQQKPGKAPKLLISAGNTLRPGVPSRFSGSGSGTDFTFTISSLQPEDIATYYCLQSDNLPYTFGGGTKLEIKRTVAAPSVFIFPPSDEQLKSGTASVVCLLNNFYPREAKVQWKVDNALQSGNSQESVTEQDSKDSTYSLSSTLTLSKADYEKHKVYACEVTHQGLSSPVTKSFNRGEC

SEQ ID NO: 124 - protein, 214 aa, synthetic construct
DIQMTQSPSSLSASVGDRVTITCVTSIDIDDDVNWYQQKPGKAPKLLISAGNTLRPGVPSRFSGSGSGTDFTFTISSLQPEDIATYYCLQSDNLPYTFGGGTKLEIKRTVAAPSVFIFPPSDEQLKSGTASVVCLLNNFYPREAKVQWKVDNALQSGNSQESVTEQDSKDSTYSLSSTLTLSKADYEKHKVYACEVTHQGLSSPVTKSFNRGEC

SEQ ID NO: 125 - protein, 214 aa, synthetic construct
DIQMTQSPSSLSASVGDRVTITCQTSIDIDDDVNWYQQKPGKAPKLLISAGNTLETGVPSRFSGSGSGTDFTFTISSLQPEDIATYYCLQSDNLPYTFGGGTKLEIKRTVAAPSVFIFPPSDEQLKSGTASVVCLLNNFYPREAKVQWKVDNALQSGNSQESVTEQDSKDSTYSLSSTLTLSKADYEKHKVYACEVTHQGLSSPVTKSFNRGEC